European Patent Application EP 4 502 167 A2, published February 5, 2025. Title: N-GLYCOSYLATION. Applicant: DTU Biosustain. The sequence listing filed with the application follows.

SEQUENCE LISTING (60 sequences)

SEQ ID NO: 1 - DNA, 39 bp, synthetic construct
  misc_feature 1..39: note = mgat1-WT
  source 1..39: mol_type = other DNA
aacaagttcaagttcccagcagctgtggtagtggaggac

SEQ ID NO: 2 - DNA, 37 bp, synthetic construct
  misc_feature 1..37: note = mgat1-alle1
  source 1..37: mol_type = other DNA
aacaagttcaagttccgcagctgtggtagtggaggac

SEQ ID NO: 3 - DNA, 54 bp, synthetic construct
  misc_feature 1..54: note = mgat2-WT
  source 1..54: mol_type = other DNA
tcctttgtcgcccattgctgctccagaggacgaagccgcaggcggccaccacga

SEQ ID NO: 4 - DNA, 49 bp, synthetic construct
  misc_feature 1..49: note = mgat2-alle1
  source 1..49: mol_type = other DNA
tcctttgtcgcccattgctgctccacgaagccgcaggcggccaccacga

SEQ ID NO: 5 - DNA, 39 bp, synthetic construct
  misc_feature 1..39: note = mgat3-WT
  source 1..39: mol_type = other DNA
ttcctggaccacttcccacccggtggccggcaggatggc

SEQ ID NO: 6 - DNA, 18 bp, synthetic construct
  misc_feature 1..18: note = mgat3-alle1
  source 1..18: mol_type = other DNA
ttcctggaccactatggc

SEQ ID NO: 7 - DNA, 20 bp, synthetic construct
  misc_feature 1..20: note = mgat3-alle2 (N-terminus)
  source 1..20: mol_type = other DNA
ttcctggaccactgataccc

SEQ ID NO: 8 - DNA, 19 bp, synthetic construct
  misc_feature 1..19: note = mgat3-alle2 (C-terminus)
  source 1..19: mol_type = other DNA
cggtggccggcaggatggc

SEQ ID NO: 9 - DNA, 60 bp, synthetic construct
  misc_feature 1..60: note = mgat4A-WT
  source 1..60: mol_type = other DNA
ttctgagttgaatgccattgtccaacagtttcgccgtgcaggagcagcaactaacggaag

SEQ ID NO: 10 - DNA, 55 bp, synthetic construct
  misc_feature 1..55: note = mgat4A-alle1
  source 1..55: mol_type = other DNA
ttctgagttgaatgccattgtccaacagccgtgcaggagcagcaactaacggaag

SEQ ID NO: 11 - DNA, 73 bp, synthetic construct
  misc_feature 1..73: note = mgat4A-alle2
  source 1..73: mol_type = other DNA
ttctgagttgaatgccattgtccaacagttgaattctagatgatcgccgtgcaggagcagcaactaacggaag

SEQ ID NO: 12 - DNA, 41 bp, synthetic construct
  misc_feature 1..41: note = mgat4B-WT
  source 1..41: mol_type = other DNA
gccctccagcagccctctgaggactggatgatcctggagtt

SEQ ID NO: 13 - DNA, 34 bp, synthetic construct
  misc_feature 1..34: note = mgat4B-alle1
  source 1..34: mol_type = other DNA
gccctccagcagccctctggatgatcctggagtt

SEQ ID NO: 14 - DNA, 38 bp, synthetic construct
  misc_feature 1..38: note = mgat4C-WT
  source 1..38: mol_type = other DNA
atacttcagactattatgtaatgctcgaagatgatgtt

SEQ ID NO: 15 - DNA, 25 bp, synthetic construct
  misc_feature 1..25: note = mgat4C-alle1
  source 1..25: mol_type = other DNA
atacttcagactcgaagatgatgtt

SEQ ID NO: 16 - DNA, 30 bp, synthetic construct
  misc_feature 1..30: note = mgat4C-alle2
  source 1..30: mol_type = other DNA
atacttcagactatgctcgaagatgatgtt

SEQ ID NO: 17 - DNA, 64 bp, synthetic construct
  misc_feature 1..64: note = mgat5-WT
  source 1..64: mol_type = other DNA
gggggatgatgcttctgcacttcaccatccagcagcggactcagcctgagagcagctccatgtt

SEQ ID NO: 18 - DNA, 78 bp, synthetic construct
  misc_feature 1..78: note = mgat5-alle1
  source 1..78: mol_type = other DNA
gggggatgatgcttctgcacttcaccatccagcatgaattctagatgagcggactcagcctgagagcagctccatgtt

SEQ ID NO: 19 - DNA, 63 bp, synthetic construct
  misc_feature 1..63: note = mgat5-alle2
  source 1..63: mol_type = other DNA
gggggatgatgcttctgcacttcaccatccagagcggactcagcctgagagcagctccatgtt

SEQ ID NO: 20 - DNA, 35 bp, synthetic construct
  misc_feature 1..35: note = mgat5-alle3 (N-terminus)
  source 1..35: mol_type = other DNA
gggggatgatgcttctgcacttcaccatccagcag

SEQ ID NO: 21 - DNA, 29 bp, synthetic construct
  misc_feature 1..29: note = mgat5-alle3 (C-terminus)
  source 1..29: mol_type = other DNA
cggactcagcctgagagcagctccatgtt

SEQ ID NO: 22 - DNA, 39 bp, synthetic construct
  misc_feature 1..39: note = mgat5B-WT
  source 1..39: mol_type = other DNA
cgtggcgccctccgcaagatgagtgacctgctggagctg

SEQ ID NO: 23 - DNA, 32 bp, synthetic construct
  misc_feature 1..32: note = mgat5B-alle1
  source 1..32: mol_type = other DNA
cagctccagcaggtcttgcggagggcgccacg

SEQ ID NO: 24 - DNA, 34 bp, synthetic construct
  misc_feature 1..34: note = mgat5B-alle2
  source 1..34: mol_type = other DNA
cagctccagcaggtatcttgcggagggcgccacg

SEQ ID NO: 25 - DNA, 39 bp, synthetic construct
  misc_feature 1..39: note = B3gnt1-WT
  source 1..39: mol_type = other DNA
tgcagctgctctacctgtcgctgctctccggactgcacg

SEQ ID NO: 26 - DNA, 50 bp, synthetic construct
  misc_feature 1..50: note = B3gnt1-alle1
  source 1..50: mol_type = other DNA
tgcagctgctctacctgtcgcagctgctctacctgtctccggactgcacg

SEQ ID NO: 27 - DNA, 34 bp, synthetic construct
  misc_feature 1..34: note = B3gnt1-alle2
  source 1..34: mol_type = other DNA
tgcagctgctctacctgtctctccggactgcacg

SEQ ID NO: 28 - DNA, 35 bp, synthetic construct
  misc_feature 1..35: note = B3gnt2-WT
  source 1..35: mol_type = other DNA
ttcagcccttcccgggcgtactggaacagagagca

SEQ ID NO: 29 - DNA, 34 bp, synthetic construct
  misc_feature 1..34: note = B3gnt2-alle1
  source 1..34: mol_type = other DNA
ttcagcccttccgggcgtactggaacagagagca

SEQ ID NO: 30 - DNA, 31 bp, synthetic construct
  misc_feature 1..31: note = B3gnt2-alle2
  source 1..31: mol_type = other DNA
ttcagcccttcccgtactggaacagagagca

SEQ ID NO: 31 - DNA, 39 bp, synthetic construct
  misc_feature 1..39: note = B4galt1-WT
  source 1..39: mol_type = other DNA
tgcatccggtcctacagcgccagcaactggactatggta

SEQ ID NO: 32 - DNA, 43 bp, synthetic construct
  misc_feature 1..43: note = B4galt1-alle1
  source 1..43: mol_type = other DNA
tgcatccggtcctacagcgccagccagcaactggactatggta

SEQ ID NO: 33 - DNA, 40 bp, synthetic construct
  misc_feature 1..40: note = B4galt2-WT
  source 1..40: mol_type = other DNA
cagccccgccactttgccatcgccatggacaagtttggct

SEQ ID NO: 34 - DNA, 18 bp, synthetic construct
  misc_feature 1..18: note = B4galt2-alle1 (N-terminus)
  source 1..18: mol_type = other DNA
cagccccgccactttgcc

SEQ ID NO: 35 - DNA, 22 bp, synthetic construct
  misc_feature 1..22: note = B4galt2-alle1 (C-terminus)
  source 1..22: mol_type = other DNA
atcgccatggacaagtttggct

SEQ ID NO: 36 - DNA, 41 bp, synthetic construct
  misc_feature 1..41: note = B4galt3-WT
  source 1..41: mol_type = other DNA
ctagccctcaagtcaggatgttgcggaggctgctggagagg

SEQ ID NO: 37 - DNA, 46 bp, synthetic construct
  misc_feature 1..46: note = B4galt3-alle1
  source 1..46: mol_type = other DNA
ctagccctcaagtcaggatgtcgtgttgcggaggctgctggagagg

SEQ ID NO: 38 - DNA, 43 bp, synthetic construct
  misc_feature 1..43: note = B4galt3-alle2
  source 1..43: mol_type = other DNA
ctagccctcaagtcaggatgttgcccggaggctgctggagagg

SEQ ID NO: 39 - DNA, 39 bp, synthetic construct
  misc_feature 1..39: note = B4galt4-WT
  source 1..39: mol_type = other DNA
aactgggactgctttatattccacgatgtggacctggtg

SEQ ID NO: 40 - DNA, 40 bp, synthetic construct
  misc_feature 1..40: note = B4galt4-alle1
  source 1..40: mol_type = other DNA
aactgggactgctttattattccacgatgtggacctggtg

SEQ ID NO: 41 - DNA, 43 bp, synthetic construct
  misc_feature 1..43: note = B4galt4-alle2
  source 1..43: mol_type = other DNA
aactgggactgctttatatttattccacgatgtggacctggtg

SEQ ID NO: 42 - DNA, 43 bp, synthetic construct
  misc_feature 1..43: note = st3Gal3-WT
  source 1..43: mol_type = other DNA
ctctctctttgtccttgctggcttcaaatggcaggacttcaag

SEQ ID NO: 43 - DNA, 38 bp, synthetic construct
  misc_feature 1..38: note = st3Gal3-alle1
  source 1..38: mol_type = other DNA
ctctctctttgtccttgctcaaatggcaggacttcaag

SEQ ID NO: 44 - DNA, 42 bp, synthetic construct
  misc_feature 1..42: note = st3Gal3-alle2
  source 1..42: mol_type = other DNA
ctctctctttgtccttgctggctcaaatggcaggacttcaag

SEQ ID NO: 45 - DNA, 43 bp, synthetic construct
  misc_feature 1..43: note = st3Gal4-WT
  source 1..43: mol_type = other DNA
ggcagcctccagtgtcgtcgttgtgttgtggtggggaatgggc

SEQ ID NO: 46 - DNA, 47 bp, synthetic construct
  misc_feature 1..47: note = st3Gal4-alle1
  source 1..47: mol_type = other DNA
ggcagcctccagtgtcgtcgttgtttgtgttgtggtggggaatgggc

SEQ ID NO: 47 - DNA, 39 bp, synthetic construct
  misc_feature 1..39: note = st3Gal4-alle2
  source 1..39: mol_type = other DNA
ggcagcctccagtgtcgtcggttgtggtggggaatgggc

SEQ ID NO: 48 - DNA, 39 bp, synthetic construct
  misc_feature 1..39: note = st3Gal6-WT
  source 1..39: mol_type = other DNA
cggtacctctgattttgctttgccctatgggacaaggcc

SEQ ID NO: 49 - DNA, 35 bp, synthetic construct
  misc_feature 1..35: note = st3Gal6-alle1
  source 1..35: mol_type = other DNA
cggtacctctgattttgcttctatgggacaaggcc

SEQ ID NO: 50 - DNA, 17 bp, synthetic construct
  misc_feature 1..17: note = st3Gal6-alle2
  source 1..17: mol_type = other DNA
cggtacctctgaaggcc

SEQ ID NO: 51 - DNA, 40 bp, synthetic construct
  misc_feature 1..40: note = fut8-WT
  source 1..40: mol_type = other DNA
caaatacttgatccgtccacaaccttggctggaaagggaa

SEQ ID NO: 52 - DNA, 39 bp, synthetic construct
  misc_feature 1..39: note = fut8-alle1
  source 1..39: mol_type = other DNA
caaatacttgatccgtccacaacctggctggaaagggaa

SEQ ID NO: 53 - DNA, 41 bp, synthetic construct
  misc_feature 1..41: note = fut8-alle2
  source 1..41: mol_type = other DNA
caaatacttgatccgtccacaacctttggctggaaagggaa

SEQ ID NO: 54 - DNA, 120 bp, synthetic construct
  misc_feature 1..120: note = ssODN with 60bp homology arm sequences
  source 1..120: mol_type = other DNA
gagagagattggtcttgcttgtcatcaccaacgtatgaaccagtgtgatggtgaaatgagtcgccgtgcaggagcagcaactaacggaagtaacactgcattgactacattttcaggtac

SEQ ID NO: 55 - DNA, 21 bp, synthetic construct
  misc_feature 1..21: note = Mgataex1F
  source 1..21: mol_type = other DNA
tatccactgtgttgcttgctg

SEQ ID NO: 56 - DNA, 21 bp, synthetic construct
  misc_feature 1..21: note = Mgataex2R
  source 1..21: mol_type = other DNA
actgctcttccagaggtcctg

SEQ ID NO: 57 - DNA, 27 bp, synthetic construct
  misc_feature 1..27: note = Mgataex2F
  source 1..27: mol_type = other DNA
gaacgccttcgaatagctgaacatagg

SEQ ID NO: 58 - DNA, 23 bp, synthetic construct
  misc_feature 1..23: note = Mgat4aEx1gRNA
  source 1..23: mol_type = other DNA
ggtataccacatggcaaaatggg

SEQ ID NO: 59 - DNA, 23 bp, synthetic construct
  misc_feature 1..23: note = Mgat4aEx2gRNA
  source 1..23: mol_type = other DNA
gtccaacagtttcgccgtgcagg

SEQ ID NO: 60 - DNA, 3873 bp, synthetic construct
  misc_feature 1..3873: note = Shuttle vector
  source 1..3873: mol_type = other DNA
tcgcgcgtttcggtgatgacggtgaaaacctctgacacatgcagctcccggagacggtcacagcttgtctgtaagcggatgccgggagcagacaagcccgtcagggcgcgtcagcgggtgttggcgggtgtcggggctggcttaactatgcggcatcagagcagattgtactgagagtgcaccatatgcggtgtgaaataccgcacagatgcgtaaggagaaaataccgcatcaggcgccattcgccattcaggctgcgcaactgttgggaagggcgatcggtgcgggcctcttcgctattacgccagctggcgaaagggggatgtgctgcaaggcgattaagttgggtaacgccagggttttcccagtcacgacgttgtaaaacgacggccagtgaattcgagctcggtaccaagcttggttgcatgctgtccggagtctcagcgttataccagaagtgacctgggtcggggaagactatagtgtcacctaaatctctagagcccttcattaggcgcgccaatcccattgcaaattctacaaaaggagtgtttcccaactgctctatcaagaggaatgttgcacactgtgacctgaatgcaaacatcacacgcgccagcagagaggaagaagagaggcttccctgaccgggaatcgaacccgggccgcggcggtgagagcgccgaatcctaaccactagaccaccagggagcacgcgccaaagctcaatgagctataattatccccttggaaaacctacaaaaacagtgtttcaaaactgctctgtgaaaagggacctttgctagcacgcggcgccaggcaaaacgtgggcacgctgcgttggccgggaatcgaacccgggtcaactgcttggaaggcagctatgctcaccactataccaccaacgcgcacacgcgccagcagattctacgggaagagtgtttcaaaactgctctatcaagagaaatgttccaccttgtgtgtggaatgcagccatcacacgcgtccatgaaagggcttaattaagatatcgtttaaacgtcgacctgcagaggccggcggataactagctgatcgcggaatcctgtccctaggccacccactgtggggtgcccttcattaggcgcgccaatcccattgcaaattctacaaaaggagtgtttcccaactgctctatcaagaggaatgttgcacactgtgacctgaatgcaaacatcacacgcgccagcagagaggaagaagagaggcttccctgaccgggaatcgaacccgggccgcggcggtgagagcgccgaatcctaaccactagaccaccagggagcacgcgccaaagctcaatgagctataattatccccttggaaaacctacaaaaacagtgtttcaaaactgctctgtgaaaagggacctttgctagcacgcggcgccaggcaaaacgtgggcacgctgcgttggccgggaatcgaacccgggtcaactgcttggaaggcagctatgctcaccactataccaccaacgcgcacacgcgccagcagattctacgggaagagtgtttcaaaactgctctatcaagagaaatgttccaccttgtgtgtggaatgcagccatcacacgcgtccatgaaagggcggttgcatgctgtccggagtctcagcgttataccagaagtgacctgggtcggggaagaaaagcttcatggtcatagctgtttcctgtgtgaaattgttatccgctcacaattccacacaacatacgagccggaagcataaagtgtaaagcctggggtgcctaatgagtgagctaactcacattaattgcgttgcgctcactgcccgctttccagtcgggaaacctgtcgtgccagctgcattaatgaatcggccaacgcgcggggagaggcggtttgcgtattgggcgctcttccgcttcctcgctcactgactcgctgcgctcggtcgttcggctgcggcgagcggtatcagctcactcaaaggcggtaatacggttatccacagaatcaggggataacgcaggaaagaacatgtgagcaaaaggccagcaaaaggccaggaaccgtaaaaaggccgcgttgctggcgtttttccataggctccgcccccctgacgagcatcacaaaaatcgacgctcaagtcagaggtggcgaaacccgacaggactataaagataccaggcgtttccccctggaagctccctcgtgcgctctcctgttccgaccctgccgcttaccggatacctgtccgcctttctcccttcgggaagcgtggcgctttctcatagctcacgctgtaggtatctcagttcggtgtaggtcgttcgctccaagctgggctgtgtgcacgaaccccccgttcagcccgaccgctgcgccttatccggtaactatcgtcttgagtccaacccggtaagacacgacttatcgccactggcagcagccactggtaacaggattagcagagcgaggtatgtaggcggtgctacagagttcttgaagtggtggcctaactacggctacactagaagaacagtatttggtatctgcgctctgctgaagccagttaccttcggaaaaagagttggtagctcttgatccggcaaacaaaccaccgctggtagcggtggtttttttgtttgcaagcagcagattacgcgcagaaaaaaaggatctcaagaagatcctttgatcttttctacggggtctgacgctcagtggaacgaaaactcacgttaagggattttggtcatgagattatcaaaaaggatcttcacctagatccttttaaattaaaaatgaagttttaaatcaatctaaagtatatatgagtaaacttggtctgacagttagaaaaactcatcgagcatcaaatgaaactgcaatttattcatatcaggattatcaataccatatttttgaaaaagccgtttctgtaatgaaggagaaaactcaccgaggcagttccataggatggcaagatcctggtatcggtctgcgattccgactcgtccaacatcaatacaacctattaatttcccctcgtcaaaaataaggttatcaagtgagaaatcaccatgagtgacgactgaatccggtgagaatggcaaaagtttatgcatttctttccagacttgttcaacaggccagccattacgctcgtcatcaaaatcactcgcatcaaccaaaccgttattcattcgtgattgcgcctgagcgagacgaaatacgcgatcgctgttaaaaggacaattacaaacaggaatcgaatgcaaccggcgcaggaacactgccagcgcatcaacaatattttcacctgaatcaggatattcttctaatacctggaatgctgttttcccagggatcgcagtggtgagtaaccatgcatcatcaggagtacggataaaatgcttgatggtcggaagaggcataaattccgtcagccagtttagtctgaccatctcatctgtaacatcattggcaacgctacctttgccatgtttcagaaacaactctggcgcatcgggcttcccatacaatcgatagattgtcgcacctgattgcccgacattatcgcgagcccatttatacccatataaatcagcatccatgttggaatttaatcgcggcctagagcaagacgtttcccgttgaatatggctcatactcttcctttttcaatattattgaagcatttatcagggttattgtctcatgagcggatacatatttgaatgtatttagaaaaataaacaaataggggttccgcgcacatttccccgaaaagtgccacctgacgtctaagaaaccattattatcatgacattaacctataaaaataggcgtatcacgaggccctttcgtc